European Patent Specification EP 3 709 899 B1, published April 22, 2026. Title: SYSTEM AND METHOD FOR LEFT ATRIAL APPENDAGE CLOSURE. Applicant: Subramaniam, Raj Tun, Zaya Quintos, Robert SureCor, Inc. Application PCT/US2018/061612. The sequence listing filed with the application follows.

SEQUENCE LISTING (1 sequence)

SEQ ID NO: 1 - protein, 15 aa, Homo sapiens
GTPGPQGIAGQRGVV